European Patent Application EP 4 379 056 A1, published June 5, 2024. Title: Microorganism with weakened activity of LacI family DNA-binding transcriptional regulator and production method of L-glutamic acid using the same. Applicant: CJ CheilJedang Corporation. The sequence listing filed with the application follows.

SEQUENCE LISTING (24 sequences)

SEQ ID NO: 1 - protein, 309 aa, synthetic construct
  REGION 1..309: note = snythetic_LacI family DNA-binding transcriptional regulator (Q310var.)
MASETSSPKKRATTLKDIAQATQLSVSTVSRALANNASIPESTRIRVVEAAQKLNYRPNAQARALRKSRTDTIGVIIPNIENPYFSSLAASIQKAAREAGVSTILSNSEENPELLGQTLAIMDDQRLDGIIVVPHIQSEEQVTDLVDRGVPVVLADRSFVNSSIPSVTSDPVPGMTEAVDLLLAADVQLGYLAGPQDTSTGQLRLNTFEKLCVDRGIVGASVYYGGYRQESGYDGIKVLIKQGANAIIAGDSMMTIGALLALHEMNLKIGEDVQLIGFDNNPIFRLQNPPLSIIDQHVQEIGKRAFEIL

SEQ ID NO: 2 - DNA, 1110 bp, synthetic construct
  misc_feature 1..1110: note = snythetic_coding gene LacI family DNA-binding transcriptionalregulator (Q310 var.)
  source 1..1110: mol_type = other DNA
atggcttccgaaacctccagcccgaagaagcgggccaccacgctcaaagacatcgcgcaagcaacacagctttcagtcagcacggtgtcccgggcattggccaacaacgcgagcattccggaatccacacgcatccgagtggttgaagccgctcaaaagctgaactaccgtcccaatgcccaagctcgtgcattgcggaagtcgaggacagacaccatcggtgtcatcattccaaacattgagaacccatatttctcctcactagcagcatcgattcaaaaagctgctcgtgaagctggggtgtccaccattttgtccaactctgaagaaaacccagagctgcttggtcagactttggcgatcatggatgaccaacgcctcgatggaatcatcgtggtgccacacattcagtcagaggaacaagtcactgacttggttgacaggggagtgccagtagtgctggcagaccgtagttttgttaactcgtctattccttcggttacctcagatccagttccgggcatgactgaagctgtggacttactcctggcagctgacgtgcaattgggctaccttgccggcccgcaggatacttccactggtcagctgcgtcttaacacttttgaaaaactatgcgtggaccgcggcatcgtcggagcatctgtctattacggtggctaccgccaagaatctggatatgacggcatcaaggtgctgatcaagcagggagccaatgcgattatcgctggtgactccatgatgaccatcggtgcgttgttggctcttcatgagatgaatttgaagatcggtgaggatgtgcagctcattgggtttgataacaacccaattttccggctgcagaatccaccgctgagcatcattgaccagcacgtacaagagatcggtaagcgtgcgtttgagattctgtagaagctgatcaatggggacaccgcgcaaaaatctgtggtgattccaacgcagctcagcatcaatggatcaacggcggtttcccaaaaggccgccgcaaaagcagcaaaagcagcccaaaaagcagccgcgaaagccgcacagaacacgcaacacgaggtgagcctagatggtgaactctga

SEQ ID NO: 3 - protein, 369 aa, synthetic construct
  REGION 1..369: note = snythetic_LacI family DNA-binding transcriptional regulator(wild)
MASETSSPKKRATTLKDIAQATQLSVSTVSRALANNASIPESTRIRVVEAAQKLNYRPNAQARALRKSRTDTIGVIIPNIENPYFSSLAASIQKAAREAGVSTILSNSEENPELLGQTLAIMDDQRLDGIIVVPHIQSEEQVTDLVDRGVPVVLADRSFVNSSIPSVTSDPVPGMTEAVDLLLAADVQLGYLAGPQDTSTGQLRLNTFEKLCVDRGIVGASVYYGGYRQESGYDGIKVLIKQGANAIIAGDSMMTIGALLALHEMNLKIGEDVQLIGFDNNPIFRLQNPPLSIIDQHVQEIGKRAFEILQKLINGDTAQKSVVIPTQLSINGSTAVSQKAAAKAAKAAQKAAAKAAQNTQHEVSLDGEL

SEQ ID NO: 4 - DNA, 1110 bp, synthetic construct
  misc_feature 1..1110: note = snythetic_gene coding LacI family DNA-binding transcriptionalregulator (wild)
  source 1..1110: mol_type = other DNA
atggcttccgaaacctccagcccgaagaagcgggccaccacgctcaaagacatcgcgcaagcaacacagctttcagtcagcacggtgtcccgggcattggccaacaacgcgagcattccggaatccacacgcatccgagtggttgaagccgctcaaaagctgaactaccgtcccaatgcccaagctcgtgcattgcggaagtcgaggacagacaccatcggtgtcatcattccaaacattgagaacccatatttctcctcactagcagcatcgattcaaaaagctgctcgtgaagctggggtgtccaccattttgtccaactctgaagaaaacccagagctgcttggtcagactttggcgatcatggatgaccaacgcctcgatggaatcatcgtggtgccacacattcagtcagaggaacaagtcactgacttggttgacaggggagtgccagtagtgctggcagaccgtagttttgttaactcgtctattccttcggttacctcagatccagttccgggcatgactgaagctgtggacttactcctggcagctgacgtgcaattgggctaccttgccggcccgcaggatacttccactggtcagctgcgtcttaacacttttgaaaaactatgcgtggaccgcggcatcgtcggagcatctgtctattacggtggctaccgccaagaatctggatatgacggcatcaaggtgctgatcaagcagggagccaatgcgattatcgctggtgactccatgatgaccatcggtgcgttgttggctcttcatgagatgaatttgaagatcggtgaggatgtgcagctcattgggtttgataacaacccaattttccggctgcagaatccaccgctgagcatcattgaccagcacgtacaagagatcggtaagcgtgcgtttgagattctgcagaagctgatcaatggggacaccgcgcaaaaatctgtggtgattccaacgcagctcagcatcaatggatcaacggcggtttcccaaaaggccgccgcaaaagcagcaaaagcagcccaaaaagcagccgcgaaagccgcacagaacacgcaacacgaggtgagcctagatggtgaactctga

SEQ ID NO: 5 - DNA, 36 bp, synthetic construct
  misc_feature 1..36: note = snythetic_1F primer
  source 1..36: mol_type = other DNA
attcgagctcggtacccgaaaacccagagctgcttg

SEQ ID NO: 6 - DNA, 31 bp, synthetic construct
  misc_feature 1..31: note = snythetic_2R primer
  source 1..31: mol_type = other DNA
cattgatcagcttctacagaatctcaaacgc

SEQ ID NO: 7 - DNA, 31 bp, synthetic construct
  misc_feature 1..31: note = snythetic_3F primer
  source 1..31: mol_type = other DNA
gcgtttgagattctgtagaagctgatcaatg

SEQ ID NO: 8 - DNA, 34 bp, synthetic construct
  misc_feature 1..34: note = snythetic_4R primer
  source 1..34: mol_type = other DNA
cgactctagaggatcccccctgtgcctgcctgcg

SEQ ID NO: 9 - DNA, 17 bp, synthetic construct
  misc_feature 1..17: note = snythetic_5F primer
  source 1..17: mol_type = other DNA
gctgctcgtgaagctgg

SEQ ID NO: 10 - DNA, 18 bp, synthetic construct
  misc_feature 1..18: note = snythetic_6R primer
  source 1..18: mol_type = other DNA
gaacccacctgagcattc

SEQ ID NO: 11 - DNA, 35 bp, synthetic construct
  misc_feature 1..35: note = snythetic_7F primer
  source 1..35: mol_type = other DNA
attcgagctcggtacccccagttcggtcacaagac

SEQ ID NO: 12 - DNA, 32 bp, synthetic construct
  misc_feature 1..32: note = snythetic_8R primer
  source 1..32: mol_type = other DNA
gctttttgggctgcttcgcttcttcgggctgg

SEQ ID NO: 13 - DNA, 32 bp, synthetic construct
  misc_feature 1..32: note = snythetic_9F primer
  source 1..32: mol_type = other DNA
ccagcccgaagaagcgaagcagcccaaaaagc

SEQ ID NO: 14 - DNA, 33 bp, synthetic construct
  misc_feature 1..33: note = snythetic_10R primer
  source 1..33: mol_type = other DNA
gactctagaggatccccggacaacgccttggcg

SEQ ID NO: 15 - DNA, 18 bp, synthetic construct
  misc_feature 1..18: note = snythetic_11F primer
  source 1..18: mol_type = other DNA
gcaaggcgatggaacgtc

SEQ ID NO: 16 - DNA, 17 bp, synthetic construct
  misc_feature 1..17: note = snythetic_12R primer
  source 1..17: mol_type = other DNA
ctcatccaagtggtgcg

SEQ ID NO: 17 - DNA, 38 bp, synthetic construct
  misc_feature 1..38: note = snythetic_13F primer
  source 1..38: mol_type = other DNA
tgaattcgagctcggtacccttgaacggaattgggtgg

SEQ ID NO: 18 - DNA, 38 bp, synthetic construct
  misc_feature 1..38: note = snythetic_14R primer
  source 1..38: mol_type = other DNA
cccaggtggcatcggtaccttcacccagcgccacgcag

SEQ ID NO: 19 - DNA, 39 bp, synthetic construct
  misc_feature 1..39: note = snythetic_15F primer
  source 1..39: mol_type = other DNA
cgctgggtgaaggtaccgatgccacctgggttggtcaag

SEQ ID NO: 20 - DNA, 38 bp, synthetic construct
  misc_feature 1..38: note = snythetic_16R primer
  source 1..38: mol_type = other DNA
gtcgactctagaggatccccggacaaggaatggagaga

SEQ ID NO: 21 - DNA, 18 bp, synthetic construct
  misc_feature 1..18: note = snythetic_17F primer
  source 1..18: mol_type = other DNA
cttaccgttgttgccctt

SEQ ID NO: 22 - DNA, 19 bp, synthetic construct
  misc_feature 1..19: note = snythetic_18R primer
  source 1..19: mol_type = other DNA
ctccttcacccacatcatt

SEQ ID NO: 23 - protein, 1205 aa, synthetic construct
  REGION 1..1205: note = snythetic_odhA protein (wild)
MFQQFQKDPKSVDKEWRELFEAQGGPNATPATTEAQPSAPKESAKPAPKAAPAAKAAPRVETKPAAKTAPKAKESSVPQQPKLPEPGQTPIRGIFKSIAKNMDISLEIPTATSVRDMPARLMFENRAMVNDQLKRTRGGKISFTHIIGYAMVKAVMAHPDMNNSYDVIDGKPTLIVPEHINLGLAIDLPQKDGSRALVVAAIKETEKMNFSEFLAAYEDIVTRSRKGKLTMDDYQGVTVSLTNPGGIGTRHSVPRLTKGQGTIIGVGSMDYPAEFQGASEDRLAELGVGKLVTITSTYDHRVIQGAVSGEFLRTMSRLLTDDSFWDEIFDAMNVPYTPMRWAQDVPNTGVDKNTRVMQLIEAYRSRGHLIADTNPLSWVQPGMPVPDHRDLDIETHSLTIWDLDRTFSVGGFGGKETMTLREVLSRLRAAYTLKVGSEYTHILDRDERTWLQDRLEAGMPKPTQAEQKYILQKLNAAEAFENFLQTKYVGQKRFSLEGAEALIPLMDSAIDTAAGQGLDEVVIGMPHRGRLNVLFNIVGKPLASIFNEFEGQMEQGQIGGSGDVKYHLGSEGQHLQMFGDGEIKVSLTANPSHLEAVNPVMEGIVRAKQDYLDKGVDGKTVVPLLLHGDAAFAGLGIVPETINLAKLRGYDVGGTIHIVVNNQIGFTTTPDSSRSMHYATDYAKAFGCPVFHVNGDDPEAVVWVGQLATEYRRRFGKDVFIDLVCYRLRGHNEADDPSMTQPKMYELITGRETVRAQYTEDLLGRGDLSNEDAEAVVRDFHDQMESVFNEVKEGGKKQAEAQTGITGSQKLPHGLETNISREELLELGQAFANTPEGFNYHPRVAPVAKKRVSSVTEGGIDWAWGELLAFGSLANSGRLVRLAGEDSRRGTFTQRHAVAIDPATAEEFNPLHELAQSKGNNGKFLVYNSALTEYAGMGFEYGYSVGNEDSVVAWEAQFGDFANGAQTIIDEYVSSGEAKWGQTSKLILLLPHGYEGQGPDHSSARIERFLQLCAEGSMTVAQPSTPANHFHLLRRHALSDLKRPLVIFTPKSMLRNKAAASAPEDFTEVTKFQSVIDDPNVADAAKVKKVMLVSGKLYYELAKRKEKDGRDDIAIVRIEMLHPIPFNRISEALAGYPNAEEVLFVQDEPANQGPWPFYQEHLPELIPNMPKMRRVSRRAQSSTATGVAKVHQLEEKQLIDEAFEA

SEQ ID NO: 24 - DNA, 3618 bp, synthetic construct
  misc_feature 1..3618: note = snythetic_gene coding odhA protein (wild)
  source 1..3618: mol_type = other DNA
atgttccagcagttccagaaggaccccaagtccgtggacaaggaatggagagaactctttgaggcgcaggggggaccaaatgctacccccgctacaacagaagcacagccttcagcgcccaaggagtctgcgaaaccagcaccaaaggctgcccctgcagccaaggcagcaccgcgcgtagaaaccaagccggccgccaagaccgcccctaaggccaaggagtcctcagtgccacagcaacctaagcttccggagccaggacaaaccccaatcaggggtattttcaagtccatcgcgaagaacatggatatctccctggaaatcccaaccgcaacctcggttcgcgatatgccagctcgcctcatgttcgaaaaccgcgcgatggtcaacgatcagctcaagcgcacccgcggtggcaagatctccttcacccacatcattggctacgccatggtgaaggcagtcatggctcacccggacatgaacaactcctacgacgtcatcgacggcaagccaaccctgatcgtgcctgagcacatcaacctgggccttgccatcgaccttcctcagaaggacggctcccgcgcacttgtcgtagcagccatcaaggaaaccgagaagatgaacttctccgagttcctcgcagcatacgaagacatcgtgacacgctcccgcaagggcaagctcaccatggatgactaccagggcgttaccgtttccttgaccaacccaggtggcatcggtacccgccactctgtcccacgtctgaccaagggccagggcaccatcatcggtgtcggttccatggattacccagcagagttccagggcgcttccgaagaccgccttgcagagctcggcgttggcaagcttgtcaccatcacctccacctacgatcaccgcgtgatccagggtgctgtgtccggtgaattcctgcgtaccatgtctcgcctgctcaccgatgattccttctgggatgagatcttcgacgcaatgaacgttccttacaccccaatgcgttgggcacaggacgttccaaacaccggtgttgataagaacacccgcgtcatgcagctcattgaggcataccgctcccgtggacacctcatcgctgacaccaacccactttcatgggttcagcctggcatgccagttccagaccaccgcgacctcgacatcgagacccacagcctgaccatctgggatctggaccgtaccttcagcgtcggtggcttcggcggcaaggagaccatgaccctgcgcgaggtactgtcccgcctgcgcgctgcctacaccttgaaggtcggctccgaatacacccacatcctggaccgcgacgagcgcacctggctgcaggaccgcctcgaagccggaatgccaaagccaacccaggcagagcagaagtacatcctgcagaagctgaacgccgcagaggctttcgagaacttcctgcagaccaagtacgtcggccagaagcgcttctccctcgaaggtgcagaagctctcatcccactgatggactccgccatcgacaccgccgcaggccagggcctcgacgaagttgtcatcggtatgccacaccgtggtcgcctcaacgtgctgttcaacatcgtgggcaagccactggcatccatcttcaacgagtttgaaggccaaatggagcagggccagatcggtggctccggtgacgtgaagtaccacctcggttccgaaggccagcacctgcagatgttcggcgacggcgagatcaaggtctccctgactgctaacccgtcccacctggaagctgttaacccagtgatggaaggtatcgtccgcgcaaagcaggactacctggacaagggcgtagacggcaagactgttgtgccactgctgctccacggtgacgctgcattcgcaggcctgggcatcgtgccagaaaccatcaacctggctaagctgcgtggctacgacgtcggaggcaccatccacatcgtggtgaacaaccagatcggcttcaccaccaccccagactccagccgctccatgcactacgcaaccgactacgccaaggcattcggctgcccagtcttccacgtcaatggtgatgacccagaggcagttgtctgggttggccagctggcaaccgagtaccgtcgtcgcttcggcaaggacgtcttcatcgacctcgtttgctaccgcctccgcggccacaacgaagctgatgatccttccatgacccagccaaagatgtatgagctcatcaccggccgcgagaccgttcgtgctcagtacaccgaagacctgctcggacgtggagacctctccaacgaagatgcagaagcagtcgtccgcgacttccacgaccagatggaatctgtgttcaacgaagtcaaggaaggcggcaagaagcaggctgaggcacagaccggcatcaccggctcccagaagcttccacacggccttgagaccaacatctcccgtgaagagctcctggaactgggacaggctttcgccaacaccccagaaggcttcaactaccacccacgtgtggctccagttgctaagaagcgcgtctcctctgtcaccgaaggtggcatcgactgggcatggggcgagctcctcgccttcggttccctggctaactccggccgcttggttcgccttgcaggtgaagattcccgccgcggtaccttcacccagcgccacgcagttgccatcgacccagcgaccgctgaagagttcaacccactccacgagcttgcacagtccaagggcaacaacggtaagttcctggtctacaactccgcactgaccgagtacgcaggcatgggcttcgagtacggctactccgtaggaaacgaagactccgtcgttgcatgggaagcacagttcggcgacttcgccaacggcgctcagaccatcatcgatgagtacgtctcctcaggcgaagctaagtggggccagacctccaagctgatccttctgctgcctcacggctacgaaggccagggcccagaccactcttccgcacgtatcgagcgcttcctgcagctgtgcgctgagggttccatgactgttgctcagccatccaccccagcaaaccacttccacctgctgcgtcgtcacgctctgtccgacctgaagcgtccactggttatcttcaccccgaagtccatgctgcgtaacaaggctgctgcctccgcaccagaagacttcactgaggtcaccaagttccaatccgtgatcgacgatccaaacgttgcagatgcagccaaggtgaagaaggtcatgctggtctccggcaagctgtactacgaattggcaaagcgcaaggagaaggacggacgcgacgacatcgcgatcgttcgtatcgaaatgctccacccaattccgttcaaccgcatctccgaggctcttgccggctaccctaacgctgaggaagtcctcttcgttcaggatgagccagcaaaccagggcccatggccgttctaccaggagcacctcccagagctgatcccgaacatgccaaagatgcgccgcgtttcccgccgcgctcagtcctccaccgcaactggtgttgctaaggtgcaccagctggaggagaagcagcttatcgacgaggctttcgaggcttaa